European Patent Application EP 4 644 565 A1, published November 5, 2025. Title: SEQUENCING METHOD. Applicant: BGI SHENZHEN. Application EP 22969635.6, filed December 29, 2022. The sequence listing filed with the application follows.

SEQUENCE LISTING (6 sequences)

SEQ ID NO: 1 - DNA, 47 bp, synthetic construct
  source 1..47: mol_type = other DNA; note = Single-stranded DNA sequence 1
ttttttttttttttttttttggttgtttctgttggtgctgatattgc

SEQ ID NO: 2 - DNA, 67 bp, synthetic construct
  source 1..67: mol_type = other DNA; note = Single-stranded DNA sequence 2
cgttatagtcgtggttgtctttgttggtttttttttttttttttttttttttttttttttttttttt

SEQ ID NO: 3 - DNA, 27 bp, synthetic construct
  source 1..27: mol_type = other DNA; note = Double-stranded DNA sequence 3-sense strand
gcaatatcagcaccaacagaaacaacc

SEQ ID NO: 4 - DNA, 27 bp, synthetic construct
  source 1..27: mol_type = other DNA; note = Double-stranded DNA sequence 3-antisense strand
ggttgtttctgttggtgctgatattgc

SEQ ID NO: 5 - DNA, 15 bp, synthetic construct
  source 1..15: mol_type = other DNA; note = Tether sequence
ttgaccgctcgcctc

SEQ ID NO: 6 - DNA, 35 bp, synthetic construct
  source 1..35: mol_type = other DNA; note = Single-stranded DNA template (Sequence 4)
ttttttttttttttttttttggttggtgtggttgg